European Patent Specification EP 3 362 481 B1, published July 8, 2026. Title: PROCEDE DE PRODUCTION DE PROTEINES ERYTHROCYTAIRES. Applicant: INSTITUT NATIONAL TRANSFUSION SANGUINE INSTITUT NATIONAL DE LA SANTE ET DE LA RECHERCHE MEDICALE (INSERM) UNIVERSITE PARIS DIDEROT PARIS 7. The sequence listing filed with the application follows.

SEQUENCE LISTING (11 sequences)

SEQ ID NO: 1 - DNA, 2549 bp, Homo sapiens
  misc_feature: RHD
ggtgttggagagaggggtgatgcctggtgctggtggaacccctgcacagagacggacacaggatgagctctaagtacccgcggtctgtccggcgctgcctgcccctctgggccctaacactggaagcagctctcattctcctcttctatttttttacccactatgacgcttccttagaggatcaaaaggggctcgtggcatcctatcaagttggccaagatctgaccgtgatggcggccattggcttgggcttcctcacctcgagtttccggagacacagctggagcagtgtggccttcaacctcttcatgctggcgcttggtgtgcagtgggcaatcctgctggacggcttcctgagccagttcccttctgggaaggtggtcatcacactgttcagtattcggctggccaccatgagtgctttgtcggtgctgatctcagtggatgctgtcttggggaaggtcaacttggcgcagttggtggtgatggtgctggtggaggtgacagctttaggcaacctgaggatggtcatcagtaatatcttcaacacagactaccacatgaacatgatgcacatctacgtgttcgcagcctattttgggctgtctgtggcctggtgcctgccaaagcctctacccgagggaacggaggataaagatcagacagcaacgatacccagtttgtctgccatgctgggcgccctcttcttgtggatgttctggccaagtttcaactctgctctgctgagaagtccaatcgaaaggaagaatgccgtgttcaacacctactatgctgtagcagtcagcgtggtgacagccatctcagggtcatccttggctcacccccaagggaagatcagcaagacttatgtgcacagtgcggtgttggcaggaggcgtggctgtgggtacctcgtgtcacctgatcccttctccgtggcttgccatggtgctgggtcttgtggctgggctgatctccgtcgggggagccaagtacctgccgtttcctcatttggctgttggattttaagcaaaagcatccaagaaaaacaaggcctgttcaaaaacaagacaacttcctctcactgttgcctgcatttgtacgtgagaaacgctcatgacagcaaagtctccaatgttcgcgcaggcactggagtcagagaaaatggagttgaatcctttctctgccactctttgaggagaatctcaccatttattatgcactgtagaatacaacaataaaatacagccatgtaccacataacaacatcttggtaaacaacagactgcatatatgatggtggtcatccagtaagctaaggttaatttattattattccttgtttttttttttttttttttttttttgagatgtagtcttactctgtcacccaggctagagtgcaatggcaccatcttggctcactgcaacctctacctcctgggttcaagcaaatctcctgcctcagcctccaaagtagctgggattacaggcacccaccacatctggctaattttttgtatttttagtaaagatggggtttcaccatgttggccaggctgatctcaaactcctgacctcaagtgatctgcccgcctcggcctcccaaagtgctggaaccacaggcctgagccactgtgcccagccttgtttgcttttttaacagataacagtgtgctcatagaaactgctttgacatgactgcaatcatgtgcttcatagaaacttaattagattataccactagagtcttcagatttttatactttttttttttgaaacggagtctcactctgtcaccaggctggagtgcagtgccgcaatctcggctcactgcaacctccgcctcccaggttcaagcaattctcctgcctcagcctcccgagtagctggaattacaagtgcgcactaccacacccagctaatttttgcatttttacttgacagggtttcaccatgttggctaggatagtttcaccaggatctcttggcctcatgatcagcctgcctcggcctcccaaagtgctgggattacaggtgtgagccaccgtgcccagcctatacttccctttttgaataccatttggtgttttgaagaattaacagctttgtgaacgtggcagtgcttgtgattcaggcttccattgagaccaaggggagaacctggttgcaggacaaacagacggacagcgtgtggcagtgtttaaatgctcttctgaaggctgatacgacagctctctgtgcactgattgcatatgcatcccaagattatattattgttttctactgctatgtgtcacactttgccaaacaggatgtggaaaatgaataagcggttttcttaggcacttcttaacagacaattggtcaaaatgaactccattgcttaagaaacacataaacaccatttagtcactgaacatagctatatgtatggttgttactatgggaaatcttgttttgccaattttctttgaaaattctggcagaccaaggttctttttgtttacataatacttgaaaaataaaaatgaacaagctaacaaacta

SEQ ID NO: 2 - DNA, 1618 bp, Homo sapiens
  misc_feature: RHCE
atcgctccctcaagccctcaagtaggtgttggagagaggggtgatgcctggtgctggtggaacccctgcacagagacggacacaggatgagctctaagtacccgcggtctgtccggcgctgcctgcccctctgggccctaacactggaagcagctctcattctcctcttctatttttttacccactatgacgcttccttagaggatcaaaaggggctcgtggcatcctatcaagtcggccaagatctgaccgtgatggcggcccttggcttgggcttcctcacctcaaatttccggagacacagctggagcagtgtggccttcaacctcttcatgctggcgcttggtgtgcagtgggcaatcctgctggacggcttcctgagccagttccctcctgggaaggtggtcatcacactgttcagtattcggctggccaccatgagtgctatgtcggtgctgatctcagcgggtgctgtcttggggaaggtcaacttggcgcagttggtggtgatggtgctggtggaggtgacagctttaggcaccctgaggatggtcatcagtaatatcttcaacacagactaccacatgaacctgaggcacttctacgtgttcgcagcctattttgggctgactgtggcctggtgcctgccaaagcctctacccaagggaacggaggataatgatcagagagcaacgatacccagtttgtctgccatgctgggcgccctcttcttgtggatgttctggccaagtgtcaactctgctctgctgagaagtccaatccaaaggaagaatgccatgttcaacacctactatgctctagcagtcagtgtggtgacagccatctcagggtcatccttggctcacccccaaaggaagatcagcatgacttatgtgcacagtgcggtgttggcaggaggcgtggctgtgggtacctcgtgtcacctgatcccttctccgtggcttgccatggtgctgggtcttgtggctgggctgatctccatcgggggagccaagtgcctgccggtgtgttgtaaccgagtgctggggattcaccacatctccgtcatgcactccatcttcagcttgctgggtctgcttggagagatcacctacattgtgctgctggtgcttcatactgtctggaacggcaatggcatgattggcttccaggtcctcctcagcattggggaactcagcttggccatcgtgatagctctcacgtctggtctcctgacaggtttgctcctaaatctcaaaatatggaaagcacctcatgtggctaaatattttgatgaccaagttttctggaagtttcctcatttggctgttggattttaagcaaaagcatccaagaaaaacaaggcctgttcaaaaacaagacaacttcctctcactgttgcctgcatttgtacgtgagaaacgctcatgacagcaaagtctccttatgtataatgaaacaaggtcagagacagatttgatattaaaaaattaaagactaaaaacttagtttaagagtcaatttaataagtttaaaataaatgtttagtttcattaggatgatgctatcaatattttcttggttacagacacattattaaagttttgggttaatttta

SEQ ID NO: 3 - DNA, 3836 bp, Homo sapiens
  misc_feature: RHAG
gttcttatcaacatctcacagcctgtgaagctctcagtgtgcctctgtcctttgccacaaacatgaggttcacattccctctcatggctatagtcctggaaattgccatgattgttttatttggattatttgttgagtatgaaacggaccagactgttctcgagcagctcaacatcaccaagccaacagacatgggcatattctttgagttatatcctctgttccaagatgtacatgttatgatatttgttgggtttggcttcctcatgaccttcctgaagaaatatggcttcagcagtgtgggtatcaacctactcgttgctgctttgggcctccagtggggcactattgtacagggaatcctgcaaagccagggacagaaatttaacattggaatcaaaaacatgataaatgcagacttcagtgcagccacagttctgatatcttttggagctgtcctgggaaaaacgagccccacccaaatgctgatgttcttatcaacatctcacagcctgtgaagctctcagtgtgcctctgtcctttgccacaaacatgaggttcacattccctctcatggctatagtcctggaaattgccatgattgttttatttggattatttgttgagtatgaaacggaccagactgttctcgagcagctcaacatcaccaagccaacagacatgggcatattctttgagttatatcctctgttccaagatgtacatgttatgatatttgttgggtttggcttcctcatgaccttcctgaagaaatatggcttcagcagtgtgggtatcaacctactcgttgctgctttgggcctccagtggggcactattgtacagggaatcctgcaaagccagggacagaaatttaacattggaatcaaaaacatgataaatgcagacttcagtgcagccacagttctgatatcttttggagctgtcctgggaaaaacgagccccacccaaatgctgatcatgacaattttagaaattgttttctttgcccacaatgaatacctggttagtgaaatatttaaggcctctgacattggagcatcaatgacgatccatgcctttggggcctactttggcttggctgtagcaggcatcttgtatcgatctggactgagaaaggggcatgaaaatgaagagtccgcatactactcagacttgtttgcaatgattgggactctctttctgtggatgttttggcccagctttaactcggccattgctgaacctggagacaaacagtgcagggccattgtaaacacgtacttctctctcgctgcctgtgtgctcacagcctttgccttctccagcctagtggagcaccgaggcaagctcaacatggttcacattcagaatgccacccttgctggaggagttgctgtgggcacttgtgcggatatggcaattcacccatttggttctatgattattgggagcattgcaggaatggtctctgtgcttggatacaagttcctgactccactttttactactaaactgaggatccatgatacatgtggggtccataacctccacggcttacctggtgtagtgggaggccttgcaggcattgtggcagtagcaatgggcgcctccaacacgtctatggccatgcaggcagctgcactgggttcctctatcggaacagcagttgttggaggtctgatgacaggtttaattctaaagttgcctctctggggacagccatctgaccagaactgctatgatgattctgtttattggaaggtccctaagacgagataacttgacaatcagttccatggacatggtgaccacagccagctggaacctgaagtctaaacaccattcctgctctccagcttcctttcccattatccagaatcaagtccaaataaacaaaaagggagtaaccaaagagagtatggaccagagtgaatagatcctaagtcccaaatggccagtgtaaaaatgtccttatgtctgatgctgtctcttgctcttcaatgattaattgaggggatgttactcataaaacagataatcaaatagatcttctccaggattcccaaaaagcttttggcagtgagtaaatacagagtaaacatgtcagtttcttaatgtagacactatgtcttcaatcccaaaaattataaaactgaaacccatgaagcaagaatagatgtgagaaatctatgtaaaaaaataattaaagaaatgcatgtgtgtaaagtagtaatatgatgattttaggtagtgctttttattttaaaaatagtctagttagtaatgttgtatccttgcatgaatattattcttaattccttttgcatgttgactatttgcaacgagctcaaatgctatctgatcaaagtctattttgcataaaatgtccaataattaaatattgttataaaataaaaaaaaaaaaaaaaaaaaaaaaaaagacattggagcatcaatgacgatccatgcctttggggcctactttggcttggctgtagcaggcatcttgtatcgatctggactgagaaaggggcatgaaaatgaagagtccgcatactactcagacttgtttgcaatgattgggactctctttctgtggatgttttggcccagctttaactcggccattgctgaacctggagacaaacagtgcagggccattgtaaacacgtacttctctctcgctgcctgtgtgctcacagcctttgccttctccagcctagtggagcaccgaggcaagctcaacatggttcacattcagaatgccacccttgctggaggagttgctgtgggcacttgtgcggatatggcaattcacccatttggttctatgattattgggagcattgcaggaatggtctctgtgcttggatacaagttcctgactccactttttactactaaactgaggatccatgatacatgtggggtccataacctccacggcttacctggtgtagtgggaggccttgcaggcattgtggcagtagcaatgggcgcctccaacacgtctatggccatgcaggcagctgcactgggttcctctatcggaacagcagttgttggaggtctgatgacaggtttaattctaaagttgcctctctggggacagccatctgaccagaactgctatgatgattctgtttattggaaggtccctaagacgagataacttgacaatcagttccatggacatggtgaccacagccagctggaacctgaagtctaaacaccattcctgctctccagcttcctttcccattatccagaatcaagtccaaataaacaaaaagggagtaaccaaagagagtatggaccagagtgaatagatcctaagtcccaaatggccagtgtaaaaatgtccttatgtctgatgctgtctcttgctcttcaatgattaattgaggggatgttactcataaaacagataatcaaatagatcttctccaggattcccaaaaagcttttggcagtgagtaaatacagagtaaacatgtcagtttcttaatgtagacactatgtcttcaatcccaaaaattataaaactgaaacccatgaagcaagaatagatgtgagaaatctatgtaaaaaaataattaaagaaatgcatgtgtgtaaagtagtaatatgatgattttaggtagtgctttttattttaaaaatagtctagttagtaatgttgtatccttgcatgaatattattcttaattccttttgcatgttgactatttgcaacgagctcaaatgctatctgatcaaagtctattttgcataaaatgtccaataattaaatattgttataaaataaaaaaaaaaaaaaaaaaaaaaaaaaa

SEQ ID NO: 4 - DNA, 4129 bp, Homo sapiens
  misc_feature: SLC14A1
acacagagcagagtggggctctgagtatataactgttaggtgcctccctccagcaccatctcctgagaagcactctcccttgtcgtggaggtgggcaaatctttatcagccactgccttctgctgccaggaagccagctagagtggtctttaaagaaaactgggcatctcctgctacttaaaatcaaaaactacctaaaataaagattataaaaaagtaaggatgaatggacggtctttgattggcggcgctggtgacgcccgtcatggtcctgtttggaaggacccttttggaactaaagctggtgacgcagcgcgcagaggcatcgcccggctaagcttggccctggcagatgggtcgcaggaacaggagccagaggaagagatagccatggaggacagccccactatggttagagtggacagccccactatggttaggggtgaaaaccaggtttcgccatgtcaagggagaaggtgcttccccaaagctcttggctatgtcaccggtgacatgaaagaacttgccaaccagcttaaagacaaacccgtggtgctccagttcattgactggattctccggggcatatcccaagtggtgttcgtcaacaaccccgtcagtggaatcctgattctggtaggacttcttgttcagaacccctggtgggctctcactggctggctgggaacagtggtctccactctgatggccctcttgctcagccaggacaggtcattaatagcatctgggctctatggctacaatgccaccctggtgggagtactcatggctgtcttttcggacaagggagactatttctggtggctgttactccctgtatgtgctatgtccatgacttgcccaattttctcaagtgcattgaattccatgctcagcaaatgggacctccccgtcttcaccctccctttcaacatggcgttgtcaatgtacctttcagccacaggacattacaatccattctttccagccaaactggtcatacctataactacagctccaaatatctcctggtctgacctcagtgccctggagttgttgaaatctataccagtgggagttggtcagatctatggctgtgataatccatggacagggggcattttcctgggagccatcctactctcctccccactcatgtgcctgcatgctgccataggatcattgctgggcatagcagcgggactcagtctttcagccccatttgaggacatctactttggactctggggtttcaacagctctctggcctgcattgcaatgggaggaatgttcatggcgctcacctggcaaacccacctcctggctcttggctgtgccctgttcacggcctatcttggagtcggcatggcaaactttatggctgaggttggattgccagcttgtacctggcccttctgtttggccacgctattgttcctcatcatgaccacaaaaaattccaacatctacaagatgcccctcagtaaagttacttatcctgaagaaaaccgcatcttctacctgcaagccaagaaaagaatggtggaaagccctttgtgagaacaagccccatttgcagccatggtcacgagtcatttctgcctgactgctccagctaacttccagggtctcagcaaactgctgtttttcacgagtatcaactttcatactgacgcgtctgtaatctgttcttatgctcattttgtattttcctttcaactccaggaatatccttgagcatatgagagtcacatccaggtgatgtgctctggtatggaatttgaaaccccaatggggccttggcactaagactggaatgtatataaagtcaaagtgctccaacagaaggaggaagtgaaaacaaactattagtatttattgatattcttggtgtttagctggctcgatgatgttaacagtattaaaaattaaaccccataaaccaactaagccttatggaattcacagtcacaaaatcgaagttaatccagaattctgtgataagcagcttggctttttttttaaatcaatgcaagttacacattatagccagaatctgtatcacagaggtgcaagctgacagcagagctcagtccccacttcctgcaaacaatggcctgcaccctatcccttgtgtgtgtgacattctctcatgggacaatgttggggtttttcagactgacaggactgcaagagggagaaaggaattttgtcaatcaaaattattctgtattgcaacttttctcagagattgcaaaggattttttaggtagagattatttttccttatgaaaaatgatctgttttaaatgagataaaataggagaagttcctggcttaacctgttcttacatattaaagaaaagttacttactgtatttatgaaatactcagcttaggcatttttactttaacccctaaattgattttgtaaatgccacaaatgcatagaattgttaccaacctccaaagggctctttaaaatcatattttttattcatttgaggatgtcttataaagactgaaggcaaaggtcagattgcttacgggtgttatttttataagttgttgaattccttaatttaaaaaagctcattattttttgcacactcacaatattctctctcagaaatcaatggcatttgaaccaccaaaaagaaataaagggctgagtgcggtggctcacgcctgtaatcccagcactttggggagcccaggcgggcagattgcttgaacccaggagttcaagaccagcctgggcagcatggtgaaaccctgtatctacaaaaaatacaaaaattagccaggcatggtggtgggtgcctgtagttccagctacttgggaggctgaggtgggaaaatgacttgagcccaggaggaggaggctgcagtgagctaagattgcaccactgcactccaacctgggcgacaagagtgaaactgtgtctctcaaaaaaaaaaaaaaacaaacaaaaacaaaaacaaaacaaaacaaaacaaaacaaaacaggtaaggattcccctgttttcctctctttaattttaaagttatcagttccgtaaagtctctgtaaccaaacatactgaagacagcaacagaagtcacgttcagggactggctcacacctgtaatcccagcactttgggagatggaggtaaaaggatctcttgagcccaggagttcaagaccagcttgggcaacatagcaagactccatctcttaaaaaataaaaatagtaacattagccaggtgtagcagcacacatctgcagcagctactcaggaggctgaggtggaaagatcgcttgtgcacagaagttcgaggctgcagtgagctatatgatcatgtcactgcactccagcctgtgtgaccgagcaagaccctatctcaaaaaaattaattaattaattaattaattaatttaaaaaggaagtcatgttcatttactttccacttcagtgtgtatcgtgtagtattttggaggttggaaagtgaaacgtaggaatcctgaagattttttccacttctagtttgcagtgctcagtgcacaatatacattttgctgaatgaataaacagaaatagggaagtaaacctacaaatattttagggagaagctcacttcttccttttctcaggaaaccaagcaagcaaacatatcgttccaattttaaaacccagtgaccaaagcctttggaactatgaatttgcaactgtcataggtttatggatattgctgtggagaagctcaattttcagtgtttgaactgaaccctttcttgttagggaacgtgtgaaagaagaattgtggggaaaaaaaagcaagcataaccaaagatcatcagcagtgaagaatctaggctgtggctgagagaaccagaggcctctaaaatggacccgagtcgatcttcagaacagggatctaccatgcaggagcttcttgtgctcacacaaatctgtaaatgggaacattgtacattgtcgaatttaaatgatattaattttctcaagctatttttgttactattttcctaaaattgaatatttgcagggagcacttatactttttcctaatgtctgtataacaaatttctatgcaagtacatgaataaattatgctcacagctca

SEQ ID NO: 5 - protein, 321 aa, Homo sapiens
  SITE (1)..(321): RhD
MSSKYPRSVRRCLPLWALTLEAALILLFYFFTHYDASLEDQKGLVASYQVGQDLTVMAAIGLGFLTSSFRRHSWSSVAFNLFMLALGVQWAILLDGFLSQFPSGKVVITLFSIRLATMSALSVLISVDAVLGKVNLAQLVVMVLVEVTALGNLRMVISNIFNTDYHMNMMHIYVFAAYFGLSVAWCLPKPLPEGTEDKDQTATIPSLSAMLGALFLWMFWPSFNSALLRSPIERKNAVFNTYYAVAVSVVTAISGSSLAHPQGKISKTYVHSAVLAGGVAVGTSCHLIPSPWLAMVLGLVAGLISVGGAKYLPFPHLAVGF

SEQ ID NO: 6 - protein, 417 aa, Homo sapiens
  SITE (1)..(417): RhCE
MSSKYPRSVRRCLPLWALTLEAALILLFYFFTHYDASLEDQKGLVASYQVGQDLTVMAALGLGFLTSNFRRHSWSSVAFNLFMLALGVQWAILLDGFLSQFPPGKVVITLFSIRLATMSAMSVLISAGAVLGKVNLAQLVVMVLVEVTALGTLRMVISNIFNTDYHMNLRHFYVFAAYFGLTVAWCLPKPLPKGTEDNDQRATIPSLSAMLGALFLWMFWPSVNSALLRSPIQRKNAMFNTYYALAVSVVTAISGSSLAHPQRKISMTYVHSAVLAGGVAVGTSCHLIPSPWLAMVLGLVAGLISIGGAKCLPVCCNRVLGIHHISVMHSIFSLLGLLGEITYIVLLVLHTVWNGNGMIGFQVLLSIGELSLAIVIALTSGLLTGLLLNLKIWKAPHVAKYFDDQVFWKFPHLAVGF

SEQ ID NO: 7 - protein, 409 aa, Homo sapiens
  SITE (1)..(409): RhAG
MRFTFPLMAIVLEIAMIVLFGLFVEYETDQTVLEQLNITKPTDMGIFFELYPLFQDVHVMIFVGFGFLMTFLKKYGFSSVGINLLVAALGLQWGTIVQGILQSQGQKFNIGIKNMINADFSAATVLISFGAVLGKTSPTQMLIMTILEIVFFAHNEYLVSEIFKASDIGASMTIHAFGAYFGLAVAGILYRSGLRKGHENEESAYYSDLFAMIGTLFLWMFWPSFNSAIAEPGDKQCRAIVNTYFSLAACVLTAFAFSSLVEHRGKLNMVHIQNATLAGGVAVGTCADMAIHPFGSMIIGSIAGMVSVLGYKFLTPLFTTKLRIHDTCGVHNLHGLPGVVGGLAGIVAVAMGASNTSMAMQAAALGSSIGTAVVGGLMTGLILKLPLWGQPSDQNCYDDSVYWKVPKTR

SEQ ID NO: 8 - protein, 445 aa, Homo sapiens
  SITE (1)..(445): UTB
MNGRSLIGGAGDARHGPVWKDPFGTKAGDAARRGIARLSLALADGSQEQEPEEEIAMEDSPTMVRVDSPTMVRGENQVSPCQGRRCFPKALGYVTGDMKELANQLKDKPVVLQFIDWILRGISQVVFVNNPVSGILILVGLLVQNPWWALTGWLGTVVSTLMALLLSQDRSLIASGLYGYNATLVGVLMAVFSDKGDYFWWLLLPVCAMSMTCPIFSSALNSMLSKWDLPVFTLPFNMALSMYLSATGHYNPFFPAKLVIPITTAPNISWSDLSALELLKSIPVGVGQIYGCDNPWTGGIFLGAILLSSPLMCLHAAIGSLLGIAAGLSLSAPFEDIYFGLWGFNSSLACIAMGGMFMALTWQTHLLALGCALFTAYLGVGMANFMAEVGLPACTWPFCLATLLFLIMTTKNSNIYKMPLSKVTYPEENRIFYLQAKKRMVESPL

SEQ ID NO: 9 - protein, 201 aa, Homo sapiens
  SITE (1)..(201): MSP1
GLKLLSNWDSVTSTFSKLREQLGPVTQEFWDNLEKETEGLRQEMSKDLEEVKAKVQPYLDDFQKKWQEEMELYRQKVEPLRAELQEGARQKLHELQEKLSPLGEEMRDRARAHVDALRTHLAPYSDELRQRLAARLEALKENGGARLAEYHAKATEHLSTLSEKAKPALEDLRQGLLPVLESFKVSFLSALEEYTKKLNTQ

SEQ ID NO: 10 - protein, 211 aa, Homo sapiens
  SITE (1)..(211): MSP1D1
GHHHHHHHDYDIPTTENLYFQGSTFSKLREQLGPVTQEFWDNLEKETEGLRQEMSKDLEEVKAKVQPYLDDFQKKWQEEMELYRQKVEPLRAELQEGARQKLHELQEKLSPLGEEMRDRARAHVDALRTHLAPYSDELRQRLAARLEALKENGGARLAEYHAKATEHLSTLSEKAKPALEDLRQGLLPVLESFKVSFLSALEEYTKKLNTQ

SEQ ID NO: 11 - protein, 278 aa, Homo sapiens
  SITE (1)..(278): MSP1E3D1
MGHHHHHHHDYDIPTTENLYFQGSTFSKLREQLGPVTQEFWDNLEKETEGLRQEMSKDLEEVKAKVQPYLDDFQKKWQEEMELYRQKVEPLRAELQEGARQKLHELQEKLSPLGEEMRDRARAHVDALRTHLAPYLDDFQKKWQEEMELYRQKVEPLRAELQEGARQKLHELQEKLSPLGEEMRDRARAHVDALRTHLAPYSDELRQRLAARLEALKENGGARLAEYHAKATEHLSTLSEKAKPALEDLRQGLLPVLESFKVSFLSALEEYTKKLNTQ